European Patent Specification EP 4 114 465 B1, published August 30, 2023. Title: Dose. Applicant: AstraZeneca AB. The sequence listing filed with the application follows.

SEQUENCE LISTING (24 sequences)

SEQ ID NO: 1 - protein, 117 aa, Artificial Sequence [sequence omitted]

SEQ ID NO: 2 - protein, 108 aa, Artificial Sequence [sequence omitted]

SEQ ID NO: 3 - protein, 5 aa, Artificial Sequence
  HCDR1
NYWIA

SEQ ID NO: 4 - protein, 17 aa, Artificial Sequence
  HCDR2
IIYPGDSDIRYSPSFQG

SEQ ID NO: 5 - protein, 8 aa, Artificial Sequence
  HCDR3
HDIEGFDY

SEQ ID NO: 6 - protein, 12 aa, Artificial Sequence
  LCDR1
RASQSVSSSFFA

SEQ ID NO: 7 - protein, 7 aa, Artificial Sequence
  LCDR2
GASSRAT

SEQ ID NO: 8 - protein, 9 aa, Artificial Sequence
  LCDR3
QQYDSSAIT

SEQ ID NO: 9 - protein, 107 aa, Artificial Sequence [sequence omitted]

SEQ ID NO: 10 - protein, 330 aa, Artificial Sequence
  Heavy chain constant region
ASTKGPSVFPLAPSSKSTSGGTAALGCLVKDYFPEPVTVSWNSGALTSGVHTFPAVLQSSGLYSLSSVVTVPSSSLGTQTYICNVNHKPSNTKVDKRVEPKSCDKTHTCPPCPAPEFEGGPSVFLFPPKPKDTLMISRTPEVTCVVVDVSHEDPEVKFNWYVDGVEVHNAKTKPREEQYNSTYRVVSVLTVLHQDWLNGKEYKCKVSNKALPASIEKTISKAKGQPREPQVYTLPPSREEMTKNQVSLTCLVKGFYPSDIAVEWESNGQPENNYKTTPPVLDSDGSFFLYSKLTVDKSRWQQGNVFSCSVMHEALHNHYTQKSLSLSPGK

SEQ ID NO: 11 - protein, 440 aa, Artificial Sequence
  Heavy chain
EVQLVQSGAEVKKPGESLKISCKGSGYIFTNYWIAWVRQMPGKGLESMGIIYPGDSDIRYSPSFQGQVTISADKSITTAYLQWSSLKASDTAMYYCARHDIEGFDYWGRGTLVTVSSASTKGPSVFPLAPSSKSTSGGTAALGCLVKDYFPEPVTVSWNSGALTSGVHTFPAVLQSSGLYSLSSVVTVPSSSLGTQTYICNVNHKPSNTKVDKRVEPKSCDKTHTCPPCPAPEFEGGPSVFLFPPKPKDTLMISRTPEVTCVVVDVSHEDPEVKFNWYVDGVEVHNAKTKPREEQYNSTYRVVSVLTVLHQDWLNGKEYKCKVSNKALPASIEKTISKAKGQPREPQVYTLPPSREEMTKNQVSLTCLVKGFYPSDIAVEWESNGQPENNYKTTPPVLDSDGSFFLYSKLTVDKSRWQQGNVFSCSVMHEALHNHYTQKS

SEQ ID NO: 12 - protein, 215 aa, Artificial Sequence
  Light chain
EIVLTQSPGTLSLSPGERATLSCRASQSVSSSFFAWYQQKPGQAPRLLIYGASSRATGIPDRLSGSGSGTDFTLTITRLEPEDFAVYYCQQYDSSAITFGQGTRLEIKRTVAAPSVFIFPPSDEQLKSGTASVVCLLNNFYPREAKVQWKVDNALQSGNSQESVTEQDSKDSTYSLSSTLTLSKADYEKHKVYACEVTHQGLSSPVTKSFNRGEC

SEQ ID NO: 13 - protein, 80 aa, Artificial Sequence
  H15D10 (VH)
EVQLVQSGAEVKKPGESLRISCKGSGYTFTNYWVAWVRQMPGKGLESMGIIYPGDSDTRYSPSFQGHVTISADKSISTAY

SEQ ID NO: 14 - protein, 108 aa, Artificial Sequence
  L8C3 (VL)
DIQMTQSPSSLSASLGDRVTITCRASQNVGNYLNWYQQKPGKAPKLLIYRASNLASGVPSRFSGSGSGTDFTLTISSLQPEDFATYYCQQMEHAPPTFGQGTKVEIKR

SEQ ID NO: 15 - protein, 108 aa, Artificial Sequence
  L16C11 (VL)
EIVLTQSPGTLSLSPGERATLSCRASQSVIGYYLAWYQQKPGQAPRLLIYSVSTLASGIPDRFSGSGSGTDFTLTISRLEPEDFAVYYCQQYYRFPITFGQGTKVEIK

SEQ ID NO: 16 - protein, 117 aa, Artificial Sequence
  H19B7 (VH)
EVQLVQSGAEVKKPGESLRISCKGSGYTFTNYWMAWVRQMPGKGLESMGIIYPSDSDTRYSPSFQGHVTISADKSISTAYLQWSSLKASDTAMYYCARHDVEGYDYWGQGTLVTVSS

SEQ ID NO: 17 - protein, 119 aa, Artificial Sequence
  QX006N (VH)
EVQLVESGGGLVQPGGSLRLSCAASGFSLSSYYMTWVRQAPGKGLEWVSVINVYGGTYYASWAKGRFTISRDNSKNTLYLQMNSLRAEDTAVYYCAREDVAVYMAIDLWGQGTLVTVSS

SEQ ID NO: 18 - protein, 111 aa, Artificial Sequence
  QX006N (VL)
AIQMTQSPSSLSASVGDRVTITCQASQSISNQLSWYQQKPGKAPKLLIYDASSLASGVPSRFSGSRSGTKFTLTISSLQPEDFATYYCLGIYGDGADDGIAFGGGTKVEIK

SEQ ID NO: 19 - protein, 5 aa, Artificial Sequence
  QX006N (HCDR1)
SYYMT

SEQ ID NO: 20 - protein, 16 aa, Artificial Sequence
  QX006N (HCDR2)
VINVYGGTYYASWAKG

SEQ ID NO: 21 - protein, 11 aa, Artificial Sequence
  QX006N (HCDR3)
EDVAVYMAIDL

SEQ ID NO: 22 - protein, 11 aa, Artificial Sequence
  QX006N (LCDR1)
QASQSISNQLS

SEQ ID NO: 23 - protein, 7 aa, Artificial Sequence
  QX006N (LCDR2)
DASSLAS

SEQ ID NO: 24 - protein, 13 aa, Artificial Sequence
  QX006N (LCDR3)
LGIYGDGADDGIA